European Patent Application EP 4 793 287 A1, published August 19, 2026. Title: 肿瘤微环境特异激活的CD47抗体. Applicant: 英脉德医疗科技（广东）有限公司. Application CN. The sequence listing filed with the application follows.

SEQUENCE LISTING (48 sequences)

SEQ ID NO: 1 - protein, 120 aa, synthetic construct
QSVKESEGGLFKPTDTLTLTCTVSGFSLSNYAINWVRQAPGNGLEWIGIINGYGMTYYASWAKSRSTITRNTSENTVTLKLTSLTAADTATYFCARDRYGSYVGYSSDIWGPGTLVTVSS

SEQ ID NO: 2 - protein, 113 aa, synthetic construct
AYDMTQTPASVEAAVGGTVTIKCQASQNISSRLAWYQQKPGQPPKLLIYGTSTLASGVPSRFRGSGSGTQFSLTISDLECADAATYYCQHGYYYSSSFTTYNAFGGGTEVVVK

SEQ ID NO: 3 - protein, 118 aa, synthetic construct
QSLEESGGDLVKPGASLTLTCTASGFSFSTSYWIYWVRQAPGKGLELIACIATGSDGSTYYASWASGRFTISKTSSTTVTLQMTSLTAADTATYFCAREAGNGVYNLWGQGTLVTVSS

SEQ ID NO: 4 - protein, 110 aa, synthetic construct
AYDMTQTPASVEVAVGGTVTIKCQASESIRNALAWYQQKPGQPPKLLISGASKLASGVASRFKGSGSATEFTLTISDLECADAATYYCQQYYSSSNVDNGFGGGTEVVVK

SEQ ID NO: 5 - protein, 118 aa, synthetic construct
QQQLEESGGDLVKPEGSLTLTCTASGFSFSSRYNMCWVRQAPGKGLEWIACIYTGSSGSTYYASWAKGRFTISKTSSTVDLKMTSLTAADTATYFCAGGSYSYRLNLWGQGTLVTVSS

SEQ ID NO: 6 - protein, 109 aa, synthetic construct
DVVMTQTPASVSTAVGGTVTIKCQASQSISNELSWYQQKPGQPPKLLIYRASTLESGVSSRFSGSGSGTEFTLTISDLECADAATYYCQATGYGDFGNAFGGGTEVVVK

SEQ ID NO: 7 - protein, 118 aa, synthetic construct
QQQLEESGGGLVKPEGSLTLTCTASGFSFSSGYDMCWVRQAPGRGLEWIACIYTRSSGGTYYASWAKGRFTISKTSSTVDLRMTSLTAADTATYFCAGGRSSYRLNLWGQGALVTVSS

SEQ ID NO: 8 - protein, 109 aa, synthetic construct
DVVMTQTPSPVEAAVGGTVTIKCQASQSISNELSWYQQKPGQPPKLLIYRASTLESGVSSRFKGSGSGTEFTLTISDLECADAATYYCQSTFYGDYGNAFGGGTEVVVK

SEQ ID NO: 9 - protein, 117 aa, synthetic construct
QSVEESEGGLFKPTDTLTLTCTISGFSLSNYDMIWVRQAPGNGLEYIGIISSRDKAGHAAWAKRRSTITRNPKENTVTLKMTSLTVADTATYFCARRFSSMHGLDIWGPGTLVTVSS

SEQ ID NO: 10 - protein, 110 aa, synthetic construct
AYDMTQTPSSVSAAVGGTVTIKCQASQSISNYLSWYQQKPGQPPKLLIYLASTLASGVPSRFKGSGSGTQFTLTISGVQCADAATYYCQQGYSSDSVDNVFGGGTEVVVK

SEQ ID NO: 11 - protein, 120 aa, synthetic construct
QVQLVESGGGVVQPGGSLRLSCAASGFTFSSGYDMCWVRQAPGKGLEWVSCIYTRSSGGTYYASWAKGRFTISRDNSKNTLYLQMNSLRAEDTAVYYCAKGRSSYRLNLWGQGTLVTVSS

SEQ ID NO: 12 - protein, 120 aa, synthetic construct
QQQLVESGGGVVQPGGSLRLSCAASGFTFSSGYDMCWVRQAPGKGLEWIACIYTRSSGGTYYASWAKGRFTISKDNSKNTLYLQMNSLRAEDTAVYYCAKGRSSYRLNLWGQGTLVTVSS

SEQ ID NO: 13 - protein, 120 aa, synthetic construct
QQQLVESGGGVVQPGGSLRLSCAASGFSFSSGYDMCWVRQAPGKGLEWIACIYTRSSGGTYYASWAKGRFTISKDNSKNTLYLQMNSLRAEDTAVYFCAKGRSSYRLNLWGQGTLVTVSS

SEQ ID NO: 14 - protein, 120 aa, synthetic construct
QQQLVESGGGVVQPGGSLRLSCAASGFSFSSGYDMCWVRQAPGKGLEWIACIYTRSSGGTYYASWAKGRFTISKDNSKNTVYLQMNSLRAEDTAVYFCAKGRSSYRLNLWGQGTLVTVSS

SEQ ID NO: 15 - protein, 109 aa, synthetic construct
DIQMTQSPSTLSASVGDRVTITCQASQSISNELSWYQQKPGKAPKLLIYRASTLESGVPSRFSGSGSGTEFTLTISSLQPDDFATYYCQSTFYGDYGNAFGGGTKVEIK

SEQ ID NO: 16 - protein, 109 aa, synthetic construct
DIQMTQSPSTLSASVGDRVTIKCQASQSISNELSWYQQKPGKAPKLLIYRASTLESGVSSRFSGSGSGTEFTLTISSLQPDDFATYYCQSTFYGDYGNAFGGGTKVEIK

SEQ ID NO: 17 - protein, 109 aa, synthetic construct
DIQMTQSPSTLSASVGDRVTIKCQASQSISNELSWYQQKPGKPPKLLIYRASTLESGVSSRFSGSGSGTEFTLTISSLQPDDFATYYCQSTFYGDYGNAFGGGTKVEIK

SEQ ID NO: 18 - protein, 6 aa, synthetic construct
SGYDMC

SEQ ID NO: 19 - protein, 18 aa, synthetic construct
CIYTRSSGGTYYASWAKG

SEQ ID NO: 20 - protein, 9 aa, synthetic construct
GRSSYRLNL

SEQ ID NO: 21 - protein, 11 aa, synthetic construct
QASQSISNELS

SEQ ID NO: 22 - protein, 7 aa, synthetic construct
RASTLES

SEQ ID NO: 23 - protein, 11 aa, synthetic construct
QSTFYGDYGNA

SEQ ID NO: 24 - protein, 17 aa, synthetic construct
CIYTSSGGTYCASWAKG

SEQ ID NO: 25 - protein, 5 aa, synthetic construct
NYAIN

SEQ ID NO: 26 - protein, 16 aa, synthetic construct
IINGYGMTYYASWAKS

SEQ ID NO: 27 - protein, 13 aa, synthetic construct
DRYGSYVGYSSDI

SEQ ID NO: 28 - protein, 11 aa, synthetic construct
QASQNISSRLA

SEQ ID NO: 29 - protein, 7 aa, synthetic construct
GTSTLAS

SEQ ID NO: 30 - protein, 15 aa, synthetic construct
QHGYYYSSSFTTYNA

SEQ ID NO: 31 - protein, 6 aa, synthetic construct
TSYWIY

SEQ ID NO: 32 - protein, 18 aa, synthetic construct
CIATGSDGSTYYASWASG

SEQ ID NO: 33 - protein, 9 aa, synthetic construct
EAGNGVYNL

SEQ ID NO: 34 - protein, 11 aa, synthetic construct
QASESIRNALA

SEQ ID NO: 35 - protein, 7 aa, synthetic construct
GASKLAS

SEQ ID NO: 36 - protein, 12 aa, synthetic construct
QQYYSSSNVDNG

SEQ ID NO: 37 - protein, 6 aa, synthetic construct
SRYNMC

SEQ ID NO: 38 - protein, 18 aa, synthetic construct
CIYTGSSGSTYYASWAKG

SEQ ID NO: 39 - protein, 9 aa, synthetic construct
GSYSYRLNL

SEQ ID NO: 40 - protein, 11 aa, synthetic construct
QASQSISNELS

SEQ ID NO: 41 - protein, 7 aa, synthetic construct
RASTLES

SEQ ID NO: 42 - protein, 11 aa, synthetic construct
QATGYGDFGNA

SEQ ID NO: 43 - protein, 5 aa, synthetic construct
NYDMI

SEQ ID NO: 44 - protein, 16 aa, synthetic construct
IISSRDKAGHAAWAKR

SEQ ID NO: 45 - protein, 10 aa, synthetic construct
RFSSMHGLDI

SEQ ID NO: 46 - protein, 11 aa, synthetic construct
QASQSISNYLS

SEQ ID NO: 47 - protein, 7 aa, synthetic construct
LASTLAS

SEQ ID NO: 48 - protein, 12 aa, synthetic construct
QQGYSSDSVDNV